European Patent Specification EP 3 636 287 B1, published December 3, 2025. Title: PET IMAGING OF HER2 EXPRESSION WITH AN RADIO-LABELED APTAMER. Applicant: INTEROLIGO CORPORAION. The sequence listing filed with the application follows.

SEQUENCE LISTING (35 sequences)

SEQ ID NO: 1 - DNA, 40 bp, Artificial Sequence
  core sequence represented by Clone No. 9-ER-N-A01_A05, wherein n is NapdU [5-(N-Naphthylcarboxyamide)-2'-deoxyuridine]
angnnagagnnngccngagngccncgnaagggcgnaacaa

SEQ ID NO: 2 - DNA, 40 bp, Artificial Sequence
  core sequence represented by Clone No. 9-ER-N-A02_B05, wherein n is NapdU [5-(N-Naphthylcarboxyamide)-2'-deoxyuridine]
nacngggcccgnnagccncnggcgcnccnncgcnngngcc

SEQ ID NO: 3 - DNA, 36 bp, Artificial Sequence
  core sequence represented by Clone No. 9-ER-N-A03_C05, wherein n is NapdU [5-(N-Naphthylcarboxyamide)-2'-deoxyuridine]
nnancaacgcacngagggcgncagcnncnnnnnagg

SEQ ID NO: 4 - DNA, 39 bp, Artificial Sequence
  core sequence represented by Clone No. 9-ER-N-A04_D05, wherein n is NapdU [5-(N-Naphthylcarboxyamide)-2'-deoxyuridine]
angnagagnnngccngagngccncgcaagggcgnaacag

SEQ ID NO: 5 - DNA, 40 bp, Artificial Sequence
  core sequence represented by Clone No. 9-ER-N-A06_E05, wherein n is NapdU [5-(N-Naphthylcarboxyamide)-2'-deoxyuridine]
nccngncccggnnnacacaagnnaaggcagccgcnggana

SEQ ID NO: 6 - DNA, 40 bp, Artificial Sequence
  core sequence represented by Clone No. 9-ER-N-B02_F05, wherein n is NapdU [5-(N-Naphthylcarboxyamide)-2'-deoxyuridine]
gncngaacaccgagannagcngaacgaacggnanggacgn

SEQ ID NO: 7 - DNA, 40 bp, Artificial Sequence
  core sequence represented by Clone No. 9-ER-N-B03_G05, wherein n is NapdU [5-(N-Naphthylcarboxyamide)-2'-deoxyuridine]
nccnggcangnncganggaggccnnngannacagcccaga

SEQ ID NO: 8 - DNA, 40 bp, Artificial Sequence
  core sequence represented by Clone No. 9-ER-N-B04_H05, wherein n is NapdU [5-(N-Naphthylcarboxyamide)-2'-deoxyuridine]
cgcgannagangaacgcacaanacccgnncngagnaaagn

SEQ ID NO: 9 - DNA, 40 bp, Artificial Sequence
  core sequence represented by Clone No. 9-ER-N-B08_A06, wherein n is NapdU [5-(N-Naphthylcarboxyamide)-2'-deoxyuridine]
gncngaacaccgagannagccgaacgaacggnanggacgn

SEQ ID NO: 10 - DNA, 40 bp, Artificial Sequence
  core sequence represented by Clone No. 9-ER-N-B09_B06, wherein n is NapdU [5-(N-Naphthylcarboxyamide)-2'-deoxyuridine]
gnnagacngaacgcacngagggccgcagccnancngaagg

SEQ ID NO: 11 - DNA, 40 bp, Artificial Sequence
  core sequence represented by Clone No. 9-ER-N-B12_C06, wherein n is NapdU [5-(N-Naphthylcarboxyamide)-2'-deoxyuridine]
angnnagagnnngccngagngccncgcaagggcgnaacaa

SEQ ID NO: 12 - DNA, 41 bp, Artificial Sequence
  core sequence represented by Clone No. 9-ER-N-C03_E06, wherein n is NapdU [5-(N-Naphthylcarboxyamide)-2'-deoxyuridine]
gncngagcancgcgnnnagccgaacgcncggngaggnagan

SEQ ID NO: 13 - DNA, 40 bp, Artificial Sequence
  core sequence represented by Clone No. 9-ER-N-C05_F06, wherein n is NapdU [5-(N-Naphthylcarboxyamide)-2'-deoxyuridine]
ncanggcangnncganggaggccnnngannacagcccaga

SEQ ID NO: 14 - DNA, 40 bp, Artificial Sequence
  core sequence represented by Clone No. 9-ER-N-C06_G06, wherein n is NapdU [5-(N-Naphthylcarboxyamide)-2'-deoxyuridine]
cnacacgaancaacnccccnccgcanacngaacancacaa

SEQ ID NO: 15 - DNA, 39 bp, Artificial Sequence
  core sequence represented by Clone No. 9-ER-N-C08_H06, wherein n is NapdU [5-(N-Naphthylcarboxyamide)-2'-deoxyuridine]
nnagcaaaangccangngcgnccngncccggnnnacagc

SEQ ID NO: 16 - DNA, 40 bp, Artificial Sequence
  core sequence represented by Clone No. 9-ER-N-C10_A07, wherein n is NapdU [5-(N-Naphthylcarboxyamide)-2'-deoxyuridine]
ngangnccccaacncagcngngaancnangcccccgccca

SEQ ID NO: 17 - DNA, 40 bp, Artificial Sequence
  core sequence represented by Clone No. 9-ER-N-D01_B07, wherein n is NapdU [5-(N-Naphthylcarboxyamide)-2'-deoxyuridine]
cngagcggnnacnacaccaccgngagaccnnagnnacaaa

SEQ ID NO: 18 - DNA, 40 bp, Artificial Sequence
  core sequence represented by Clone No. 9-ER-N-D02_C07, wherein n is NapdU [5-(N-Naphthylcarboxyamide)-2'-deoxyuridine]
annagangaaagcgcannccaacaacaganaancngaggg

SEQ ID NO: 19 - DNA, 40 bp, Artificial Sequence
  core sequence represented by Clone No. 9-ER-N-D04_E07, wherein n is NapdU [5-(N-Naphthylcarboxyamide)-2'-deoxyuridine]
nnnggagngncnnacggnnggagnaancgaggangganga

SEQ ID NO: 20 - DNA, 40 bp, Artificial Sequence
  core sequence represented by Clone No. 9-ER-N-D05_F07, wherein n is NapdU [5-(N-Naphthylcarboxyamide)-2'-deoxyuridine]
ccgnnaccnaccnccncgaccgngggngcccnnagnccca

SEQ ID NO: 21 - DNA, 39 bp, Artificial Sequence
  core sequence represented by Clone No. 9-ER-N-D06_G07, wherein n is NapdU [5-(N-Naphthylcarboxyamide)-2'-deoxyuridine]
nccnggcangnncganggaggccnnngannacagccaga

SEQ ID NO: 22 - DNA, 40 bp, Artificial Sequence
  core sequence represented by Clone No. 9-ER-N-D07_H07, wherein n is NapdU [5-(N-Naphthylcarboxyamide)-2'-deoxyuridine]
ccgnnaccnaccnccncgaccgngggngccnnnagnccca

SEQ ID NO: 23 - DNA, 40 bp, Artificial Sequence; identical to SEQ ID NO: 11
  core sequence represented by Clone No. 9-ER-N-D09_A08, wherein n is NapdU [5-(N-Naphthylcarboxyamide)-2'-deoxyuridine]

SEQ ID NO: 24 - DNA, 40 bp, Artificial Sequence
  core sequence represented by Clone No. 9-ER-N-D11_B08, wherein n is NapdU [5-(N-Naphthylcarboxyamide)-2'-deoxyuridine]
nccnggcangnncganggaggccnnngannacagcccagn

SEQ ID NO: 25 - DNA, 40 bp, Artificial Sequence
  core sequence represented by Clone No. 9-ER-N-E04_D08, wherein n is NapdU [5-(N-Naphthylcarboxyamide)-2'-deoxyuridine]
annagangaaagcacannccaacaacaganaancngaggg

SEQ ID NO: 26 - DNA, 40 bp, Artificial Sequence
  core sequence represented by Clone No. 9-ER-N-E11_F08, wherein n is NapdU [5-(N-Naphthylcarboxyamide)-2'-deoxyuridine]
angnnagagnnngccngagngcgncgcaagggcgnaacag

SEQ ID NO: 27 - DNA, 39 bp, Artificial Sequence
  core sequence represented by Clone No. 9-ER-N-E12_G08, wherein n is NapdU [5-(N-Naphthylcarboxyamide)-2'-deoxyuridine]
ngagaagggcngngccnnacncaaaannngggancngaa

SEQ ID NO: 28 - DNA, 40 bp, Artificial Sequence
  core sequence represented by Clone No. 9-ER-N-F05_D09, wherein n is NapdU [5-(N-Naphthylcarboxyamide)-2'-deoxyuridine]
nccnggnangnncganggaggccnnngannacagcccaga

SEQ ID NO: 29 - DNA, 40 bp, Artificial Sequence
  core sequence represented by Clone No. 9-ER-N-F08_E09, wherein n is NapdU [5-(N-Naphthylcarboxyamide)-2'-deoxyuridine]
nagancncngannaggnagaacgcccnacncnaacggcag

SEQ ID NO: 30 - DNA, 40 bp, Artificial Sequence
  core sequence represented by Clone No. 9-ER-N-F09_F09, wherein n is NapdU [5-(N-Naphthylcarboxyamide)-2'-deoxyuridine]
ngagaagggcngngccnnacncaaaannnggggancngaa

SEQ ID NO: 31 - DNA, 40 bp, Artificial Sequence; identical to SEQ ID NO: 30
  core sequence represented by Clone No. 9-ER-N-F11_G09, wherein n is NapdU [5-(N-Naphthylcarboxyamide)-2'-deoxyuridine]

SEQ ID NO: 32 - DNA, 40 bp, Artificial Sequence
  core sequence represented by Clone No. 9-ER-N-G04_B10, wherein n is NapdU [5-(N-Naphthylcarboxyamide)-2'-deoxyuridine]
cgnccnnggngagnnngggncngagcaggagcacgngagn

SEQ ID NO: 33 - DNA, 40 bp, Artificial Sequence; identical to SEQ ID NO: 25
  core sequence represented by Clone No. 9-ER-N-H01_E10, wherein n is NapdU [5-(N-Naphthylcarboxyamide)-2'-deoxyuridine]

SEQ ID NO: 34 - DNA, 40 bp, Artificial Sequence; identical to SEQ ID NO: 25
  core sequence represented by Clone No. 9-ER-N-H03_G10, wherein n is NapdU [5-(N-Naphthylcarboxyamide)-2'-deoxyuridine]

SEQ ID NO: 35 - DNA, 40 bp, Artificial Sequence
  core sequence represented by Clone No. 9-ER-N-H09_B11, wherein n is NapdU [5-(N-Naphthylcarboxyamide)-2'-deoxyuridine]
angnnagagncngccngagngccncgcaagggcgnaacag